European Patent Application EP 4 652 998 A1, published November 26, 2025. Title: Methods for treating receptor-interacting protein kinase 1-mediated disease with eclitasertib. Applicant: Technische Universität München. Application EP. The sequence listing filed with the application follows.

SEQUENCE LISTING (28 sequences)

SEQ ID NO: 1 - DNA, 20 bp, synthetic construct
  source 1..20: mol_type = other DNA
gtaacccgttgaaccccatt

SEQ ID NO: 2 - DNA, 20 bp, synthetic construct
  source 1..20: mol_type = other DNA
ccatccaatcggtagtagcg

SEQ ID NO: 3 - DNA, 20 bp, synthetic construct
  source 1..20: mol_type = other DNA
cttgacttgcagctgagcac

SEQ ID NO: 4 - DNA, 20 bp, synthetic construct
  source 1..20: mol_type = other DNA
cagagtcacccatctcagca

SEQ ID NO: 5 - DNA, 21 bp, synthetic construct
  source 1..21: mol_type = other DNA
gagtgtggagaccatcaagga

SEQ ID NO: 6 - DNA, 24 bp, synthetic construct
  source 1..24: mol_type = other DNA
tggacattcaagtcagttaccgaa

SEQ ID NO: 7 - DNA, 21 bp, synthetic construct
  source 1..21: mol_type = other DNA
tgttgtagcaaaccctcaagc

SEQ ID NO: 8 - DNA, 20 bp, synthetic construct
  source 1..20: mol_type = other DNA
atgaggtacaggccctctga

SEQ ID NO: 9 - DNA, 20 bp, synthetic construct
  source 1..20: mol_type = other DNA
aagcccttgctgtagtggtg

SEQ ID NO: 10 - DNA, 20 bp, synthetic construct
  source 1..20: mol_type = other DNA
gaagctgatggccctaaaca

SEQ ID NO: 11 - DNA, 22 bp, synthetic construct
  source 1..22: mol_type = other DNA
aatgctgactcaaaggagacga

SEQ ID NO: 12 - DNA, 21 bp, synthetic construct
  source 1..21: mol_type = other DNA
ttctgaaggcttgcatcttgc

SEQ ID NO: 13 - DNA, 21 bp, synthetic construct
  source 1..21: mol_type = other DNA
gagtgcaaggaaccccagtag

SEQ ID NO: 14 - DNA, 21 bp, synthetic construct
  source 1..21: mol_type = other DNA
ggtggatagtcccttggttgg

SEQ ID NO: 15 - DNA, 20 bp, synthetic construct
  source 1..20: mol_type = other DNA
aacctccagtctcagcacca

SEQ ID NO: 16 - DNA, 23 bp, synthetic construct
  source 1..23: mol_type = other DNA
gagagaggtactccttgaatgcc

SEQ ID NO: 17 - DNA, 22 bp, synthetic construct
  source 1..22: mol_type = other DNA
ttgttcaaggcttccccatgtt

SEQ ID NO: 18 - DNA, 22 bp, synthetic construct
  source 1..22: mol_type = other DNA
cactttcactgcttttacccca

SEQ ID NO: 19 - DNA, 20 bp, synthetic construct
  source 1..20: mol_type = other DNA
cagaccacgcaaggagttca

SEQ ID NO: 20 - DNA, 20 bp, synthetic construct
  source 1..20: mol_type = other DNA
tcttcagggaggctaccact

SEQ ID NO: 21 - DNA, 20 bp, synthetic construct
  source 1..20: mol_type = other DNA
accggaaggaaccatctcac

SEQ ID NO: 22 - DNA, 21 bp, synthetic construct
  source 1..21: mol_type = other DNA
ggcaaaactgcaccttcacac

SEQ ID NO: 23 - DNA, 21 bp, synthetic construct
  source 1..21: mol_type = other DNA
gctctctgcaaccagttctct

SEQ ID NO: 24 - DNA, 22 bp, synthetic construct
  source 1..22: mol_type = other DNA
tcgcttggttaggaagatgaca

SEQ ID NO: 25 - DNA, 20 bp, synthetic construct
  source 1..20: mol_type = other DNA
ggtaccatgaaggtctccgc

SEQ ID NO: 26 - DNA, 20 bp, synthetic construct
  source 1..20: mol_type = other DNA
ggtgtccgaggaatatgggg

SEQ ID NO: 27 - DNA, 20 bp, synthetic construct
  source 1..20: mol_type = other DNA
tttgctcctggctgctttga

SEQ ID NO: 28 - DNA, 22 bp, synthetic construct
  source 1..22: mol_type = other DNA
agcagtcaaagttgcttgcttc